European Patent Application EP 4 582 454 A1, published July 9, 2025. Title: IMMUNE CELL HAVING MEMBRANE-BOUND IL-21, AND PREPARATION METHOD THEREFOR AND USE THEREOF. Applicant: NEUKIO BIOTHERAPEUTICS (SHANGHAI) CO., LTD. The sequence listing filed with the application follows.

SEQUENCE LISTING (9 sequences)

SEQ ID NO: 1 - protein, 249 aa, synthetic construct
  source 1..249: note = Recombinant protein mb-IL21
MRSSPGNMERIVICLMVIFLGTLVHKSSSQGQDRHMIRMRQLIDIVDQLKNYVNDLVPEFLPAPEDVETNCEWSAFSCFQKAQLKSANTGNNERIINVSIKKLKRKPPSTNAGRRQKHRLTCPSCDSYEKKPPKEFLERFKSLLQKMIHQHLSSRTHGSEDSGGGGSPAPRPPTPAPTIASQPLSLRPEACRPAAGGAVHTRGLDFACDIYIWAPLAGTCGVLLLSLVITLYCNHRNRRRVCKCPRPVV

SEQ ID NO: 2 - protein, 246 aa, synthetic construct
  source 1..246: note = Recombinant protein mb-IL21
MALPVTALLLPLALLLHAARPHKSSSQGQDRHMIRMRQLIDIVDQLKNYVNDLVPEFLPAPEDVETNCEWSAFSCFQKAQLKSANTGNNERIINVSIKKLKRKPPSTNAGRRQKHRLTCPSCDSYEKKPPKEFLERFKSLLQKMIHQHLSSRTHGSEDSGGGGSPAPRPPTPAPTIASQPLSLRPEACRPAAGGAVHTRGLDFACDIYIWAPLAGTCGVLLLSLVITLYCNHRNRRRVCKCPRPVV

SEQ ID NO: 3 - protein, 24 aa, Homo sapiens
MRSSPGNMERIVICLMVIFLGTLV

SEQ ID NO: 4 - protein, 21 aa, Homo sapiens
MALPVTALLLPLALLLHAARP

SEQ ID NO: 5 - protein, 17 aa, Homo sapiens
MWLQSLLLLGTVACSIS

SEQ ID NO: 6 - protein, 21 aa, Homo sapiens
MGGLEPCSRLLLLPLLLAVSG

SEQ ID NO: 7 - protein, 16 aa, Homo sapiens
MWQLLLPTALLLLVSA

SEQ ID NO: 8 - protein, 19 aa, Homo sapiens
MLQTKDLIWTLFFLGTAVS

SEQ ID NO: 9 - protein, 20 aa, Homo sapiens
MTSKLAVALLAAFLISAALC